European Patent Specification EP 3 395 366 B1, published November 22, 2023. Title: Drug Design Method, Obtained Drug and Application Thereof. Applicant: Hefei Lifeon Pharmaceutical Co. Ltd. The sequence listing filed with the application follows.

SEQUENCE LISTING (17 sequences)

SEQ ID NO: 1 - protein, 117 aa, Artificial
  B5 VH
EVQLLESGGGLVQPGGSLRLSCAASGFTFSSYAMSWVRQAPGKGLEWVSRISPSGSSTYYADSVKGRFTISRDNSKNTLYLQMNSLRAEDTAVYYCARHTAPLFDYWGQGTLVTVSS

SEQ ID NO: 2 - protein, 108 aa, Artificial
  B5 VL
EIVLTQSPGTLSLSPGERATLSCRASQSVSSSYLAWYQQKPGQAPRLLIYKASNLATGIPDRFSGSGSGTDFTLTISRLEPEDFAVYYCQQGRHTPPTFGQGTKVEIK

SEQ ID NO: 3 - protein, 241 aa, Artificial
  B5-ScFv fusion
EVQLLESGGGLVQPGGSLRLSCAASGFTFSSYAMSWVRQAPGKGLEWVSRISPSGSSTYYADSVKGRFTISRDNSKNTLYLQMNSLRAEDTAVYYCARHTAPLFDYWGQGTLVTVSSGGGGSGGGGSGGGGSSEIVLTQSPGTLSLSPGERATLSCRASQSVSSSYLAWYQQKPGQAPRLLIYKASNLATGIPDRFSGSGSGTDFTLTISRLEPEDFAVYYCQQGRHTPPTFGQGTKVEIK

SEQ ID NO: 4 - protein, 229 aa, Artificial
  IgG4 Fc
ESKYGPPCPPCPAPEFLGGPSVFLFPPKPKDTLMISRTPEVTCVVVDVSQEDPEVQFNWYVDGVEVHNAKTKPREEQFNSTYRVVSVLTVLHQDWLNGKEYKCKVSNKGLPSSIEKTISKAKGQPREPQVYTLPPSQEEMTKNQVSLTCLVKGFYPSDIAVEWESNGQPENNYKTTPPVLDSDGSFFLYSRLTVDKSRWQEGNVFSCSVMHEALHNHYTQKSLSLSLGK

SEQ ID NO: 5 - protein, 473 aa, Artificial
  B5-Fc fusion
EVQLLESGGGLVQPGGSLRLSCAASGFTFSSYAMSWVRQAPGKGLEWVSRISPSGSSTYYADSVKGRFTISRDNSKNTLYLQMNSLRAEDTAVYYCARHTAPLFDYWGQGTLVTVSSGGGGSGGGGSGGGGSSEIVLTQSPGTLSLSPGERATLSCRASQSVSSSYLAWYQQKPGQAPRLLIYKASNLATGIPDRFSGSGSGTDFTLTISRLEPEDFAVYYCQQGRHTPPTFGQGTKVEIKAAAESKYGPPCPPCPAPEFLGGPSVFLFPPKPKDTLMISRTPEVTCVVVDVSQEDPEVQFNWYVDGVEVHNAKTKPREEQFNSTYRVVSVLTVLHQDWLNGKEYKCKVSNKGLPSSIEKTISKAKGQPREPQVYTLPPSQEEMTKNQVSLTCLVKGFYPSDIAVEWESNGQPENNYKTTPPVLDSDGSFFLYSRLTVDKSRWQEGNVFSCSVMHEALHNHYTQKSLSLSLGK

SEQ ID NO: 6 - protein, 391 aa, Artificial
  B5-IL2 fusion
EVQLLESGGGLVQPGGSLRLSCAASGFTFSSYAMSWVRQAPGKGLEWVSRISPSGSSTYYADSVKGRFTISRDNSKNTLYLQMNSLRAEDTAVYYCARHTAPLFDYWGQGTLVTVSSGGGGSGGGGSGGGGSSEIVLTQSPGTLSLSPGERATLSCRASQSVSSSYLAWYQQKPGQAPRLLIYKASNLATGIPDRFSGSGSGTDFTLTISRLEPEDFAVYYCQQGRHTPPTFGQGTKVEIKAAASSSGSSSSGSSSSGAPTSSSTKKTQLQLEHLLLDLQMILNGINNYKNPKLTRMLTFKFYMPKKATELKHLQCLEEELKPLEEVLNLAQSKNFHLRPRDLISNINVIVLELKGSETTFMCEYADETATIVEFLNRWITFCQSIISTLT

SEQ ID NO: 7 - protein, 16 aa, Artificial
  linker
GGGGSGGGGSGGGGSS

SEQ ID NO: 8 - protein, 17 aa, Artificial
  linker
AAASSSGSSSSGSSSSG

SEQ ID NO: 9 - protein, 133 aa, Artificial [sequence omitted]

SEQ ID NO: 10 - protein, 91 aa, Homo sapiens
  ED-B
EVPQLTDLSFVDITDSSIGLRWTPLNSSTIIGYRITVVAAGEGIPIFEDFVDSSVGYYTVTGLEPGIDYDISVITLINGGESAPTTLTQQT

SEQ ID NO: 11 - protein, 5 aa, Artificial
  linker
GGGGS

SEQ ID NO: 12 - protein, 6 aa, Artificial
  linker
GGGGGG

SEQ ID NO: 13 - protein, 8 aa, Artificial
  linker
GGGGGGGG

SEQ ID NO: 14 - protein, 5 aa, Artificial
  linker
EAAAK

SEQ ID NO: 15 - protein, 7 aa, Artificial
  linker
AEAAAKA

SEQ ID NO: 16 - protein, 2 aa, Artificial
  linker
AP

SEQ ID NO: 17 - protein, 2 aa, Artificial
  linker
  misc_feature (1)..(1): Xaa can be any naturally occurring amino acid, preferably Ala, Lys or Glu
XP